European Patent Specification EP 3 679 133 B1, published November 6, 2024. Title: Leistungsverbesserte Proteasevarianten I. Applicant: Henkel AG & Co. KGaA. The sequence listing filed with the application follows.

SEQUENCE LISTING (25 sequences)

SEQ ID NO: 1 - protein, 275 aa, Bacillus pumilus
AQTVPYGIPQIKAPAVHAQGYKGANVKVAVLDTGIHAAHPDLNVAGGASFVPSEPNATQDFQSHGTHVAGTIAALDNTIGVLGVAPSASLYAVKVLDRNGDGQYSWIISGIEWAVANNMDVINMSLGGPNGSTALKNAVDTANNRGVVVVAAAGNSGSTGSTSTVGYPAKYDSTIAVANVNSSNVRNSSSSAGPELDVSAPGTSILSTVPSSGYTSYTGTSMASPHVAGAAALILSKNPNLSNSQVRQRLENTATPLGNSFYYGKGLINAQAASN

SEQ ID NO: 2 - protein, 275 aa, Artificial Sequence
  Mutante 2
AQTVPYGITQIKAPAVHAQGYKGANVKVAVLDTGIHAAHPDLNVAGGASFVPSEPNATQDFQSHGTHVAGTIAALDNTIGVLGVAPSASLYAVKVLDRNGDGQYSWIISGIEWAVANNMDVINMSLGGPNGSRALKNAVDTANNRGVVVVAAAGNSGSTGSTSTVGYPAKYDSTIAVANVNSSNVRNSSSSAGPELDVSAPGTSILSTVPSSGYTCYTGTSMAAPHVAGAAALILSKNPNLSNSQVRQRLENTATPLGNSFYYGKGLINAEAASN

SEQ ID NO: 3 - protein, 275 aa, Artificial Sequence
  Mutante 3
AQTVPYGITQIKAPAVHAQGYKGANVKVAVLDTGIHAAHPDLNVAGGVSFVPSEPNATQDFQSHGTHVAGTIAALDNTIGVLGVAPSASLYAVKVLDRNGDGQYSWIISGIEWAVANNMDVINMSLGGPNSSRALKNAVDTANNRGVVVVAAAGNSGSTGSTSTVGYPAKYDSTIAVANVNSSNVRNSSSSAGPELDVSAPGTSILSTVPSSGYTCYTGTSMAAPHVAGAAALILSKNPNLSNSQVRQRLENTATPLGNSFYYGKGLINAEAASN

SEQ ID NO: 4 - protein, 275 aa, Artificial Sequence
  Mutante 4
AQTVPYGITQIKAPAVHAQGYKGANVKVAVLDTGIHAAHPDLNVAGGASFVPSEPNATQDFQSHGTHVAGTIAALDNTIGVLGVAPSASLYAVKVLDRNGDGQYSWIISGIEWAVANNMDVINMSLGGPNDSRALKNAVDTANNRGVVVVAAAGNSGSTGSTSTVGYPAKYDSTIAVANVNSSNVRNSSSSAGPELDVSAPGTSILSTVPSSGYTCYTGTSMAAPHVAGAAALILSKNPNLSNSQVRQRLENTATPLGNSFYYGKGLINAEAASN

SEQ ID NO: 5 - protein, 275 aa, Artificial Sequence
  Mutante 5
AQTVPYGITQIKAPAVHAQGYKGANVKVAVLDTGIHAAHPDLNVAGGASFVPSEPNATQDFQSHGTHVAGTIAALDNTIGVLGVAPSASLYAVKVLDRNGDGQYSWIISGIEWAVANNMDVINMSLGGPDNSKALKNAVDTANKRGVVVVAAAGNSGSTGSTSTVGYPAKYDSTIAVANVNSSNVRNSSSSAGPELDVSAPGTSILSTVPSSGYTCYTGTSMASPHVAGAAALILSKNPNLSNSQVRQRLENTATPLGNSFYYGKGLINAEAASN

SEQ ID NO: 6 - protein, 275 aa, Artificial Sequence
  Mutante 6
AQTVPYGITQIKAPAVHAQGYKGANVKVGVLDTGIHAAHPDLNVAGGASFVPSEPNATQDFQSHGTHVAGTIAALDNTIGVLGVAPSASLYAVKVLDRNGDGQYSWIISGIEWAVANNMDVINMSLGGPDNSRALKNAVDTANNRGVVVVAAAGNSGSTGSTSTVGYPAKYDSTIAVANVNSSNVRNSSSSAGPELDVSAPGTSILSTVPSSGYTCYTGTSMASPHVAGAAALILSKNPNLSNSQVRQRLENTATPLGNSFYYGKGLINAEAASN

SEQ ID NO: 7 - protein, 275 aa, Artificial Sequence
  Mutante 7
AQTVPYGITQIKAPAVHAQGYKGANVKVAVLDTGIHAAHPDLNVAGGASFVPSEPNATQDFQSHGTHVAGTIAALDNTIGVLGVAPSASLYAVKVLDRNGDGQYSWIISGIEWAVANNMDVINMSLGGPDSSKALKNAVDTANNRGVVVVAAAGNSGSTGSTSTVGYPAKYDSTIAVANVNSSNVRNSSSSAGPELDVSAPGTSILSTVPSSGYTCYTGTSMAAPHVAGAAALILSKNPNLSNSQVRQRLENTATPLGNSFYYGKGLINAEAASN

SEQ ID NO: 8 - protein, 275 aa, Artificial Sequence
  Mutante 8
AQTVPYGITQIKAPAVHAQGYKGANVKVAVLDTGIHAAHPDLNVAGGASFVPSEPNATQDFQSHGTHVAGTIAALDNTIGVLGVAPSASLYAVKVLDRNGDGQYSWIISGIEWAVANNMDVINMSLGGPDNSKALKNAVDTANLRGVVVVAAAGNSGSTGSTSTVGYPAKYDSTIAVANVNSSNVRNSSSSAGPELDVSAPGTSILSTVPSSGYTCYTGTSMASPHVAGAAALILSKNPNLSNSQVRQRLESTATPLGNSFYYGKGLINAEAASN

SEQ ID NO: 9 - protein, 275 aa, Artificial Sequence
  Mutante 9
AQTVPYGITQIKAPAVHAQGYKGANVKVAVLDTGIHAAHPDLNVAGGASFVPSEPNATQDFQSHGTHVAGTIAALDNTIGVLGVAPSASLYAVKVLDRNGDGQYSWIISGIEWAVANNMDVINMSLGGPNSSTALKNAVDTANKRGVVVVAAAGNSGSTGSTSTVGYPAKYDSTIAVANVNSSNVRNSSSSAGPELDVSAPGTSILSTVPSSGYTCYTGTSMATPHVAGAAALILSKNPNLSNSQVRQRLENTATPLGNSFYYGKGLINAEAASN

SEQ ID NO: 10 - protein, 275 aa, Artificial Sequence
  Mutante 10
AQTVPYGITQIKAPAVHAQGYKGANVKVAVLDTGIHAAHPDLNVAGGASFVPSEPNATQDFQSHGTHVAGTIAALDNTIGVLGVAPSASLYAVKVLDRNGDGQYSWIISGIEWAVANNMDVINMSLGGPSSSYALKNAVDTANLRGVVVVAAAGNSGSTGSTSTVGYPAKYDSTIAVANVNSSNVRNSSSSAGPELDVSAPGTSILSTVPSSGYTCYTGTSMAAPHVAGAAALILSKNPNLSNSQVRQRLENTATPLGNSFYYGKGLINAEAASN

SEQ ID NO: 11 - protein, 275 aa, Artificial Sequence
  Mutante 11
AQTVPYGITQIKAPAVHAQGYKGANVKVAVLDTGIHAAHPDLNVAGGASFVPSEPNATQDFQSHGTHVAGTIAALDNTIGVLGVAPSASLYAVKVLDRNGEGQYSWIISGIEWAVANNMDVINMSLGGPNNSTALKNAVDTANNRGVVVVAAAGNSGSTGSTSTVGYPAKYDSTIAVANVNSSNVRNSSSSAGPELDVSAPGTSILSTVPSSGYTCYTGTSMAAPHVAGAAALILSKNPNLSNSQVRQRLENTATPLGNSFYYGKGLINAEAASN

SEQ ID NO: 12 - protein, 275 aa, Artificial Sequence
  Mutante 12
AQTVPYGITQIKAPAVHAQGYKGANVKVAVLDTGIHAAHPDLNVAGGASFVPSEPNATQDFQSHGTHVAGTIAALDNTIGVLGVAPSASLYAVKVLDRNGDGQYSWIISGIEWAVANNMDVINMSLGGPHSSTALKNAVDTANNRGVVVVAAAGNSGSTGSTSTVGYPAKYDSTIAVANVNSSNVRNSSSSAGPELDVSAPGTSILSTVPSSGYTCYTGTSMAAPHVAGAAALILSKNPNLSNSQVRQRLENTATPLGNSFYYGKGLINAEAASN

SEQ ID NO: 13 - protein, 275 aa, Artificial Sequence
  Mutante 1
AQTVPYGITQIKAPAVHAQGYKGANVKVAVLDTGIHAAHPDLNVAGGASFVPSEPNATQDFQSHGTHVAGTIAALDNTIGVLGVAPSASLYAVKVLDRNGDGQYSWIISGIEWAVANNMDVINMSLGGPNGSTALKNAVDTANNRGVVVVAAAGNSGSTGSTSTVGYPAKYDSTIAVANVNSSNVRNSSSSAGPELDVSAPGTSILSTVPSSGYTCYTGTSMASPHVAGAAALILSKNPNLSNSQVRQRLENTATPLGNSFYYGKGLINAEAASN

SEQ ID NO: 14 - protein, 275 aa, Artificial Sequence
  Mutante 13
AQTVPYGITQIKAPAVHAQGYKGANVKVAVLDTGIHAAHPDLNVAGGASFVPSEPNATQDFQSHGTHVAGTIAALDNTIGVLGVAPSASLYAVKVLDRNGDGQYSWIISGIEWAVANNMDVINMSLGGPNGSTALKNAVDTANNRGVVVVAAAGNSGSTGSTSTVGYPAKYDSTIAVANVNSSNVRNSSSSAGPELDVSAPGTSILSTVPSSGYTSYTGTSMASPHVAGAAALILSKNPNLSNSQVRQRLENTATPLGNSFYYGKGLINAEAASN

SEQ ID NO: 15 - protein, 275 aa, Artificial Sequence
  Mutante 14
AQTVPYGIPQIKAPAVHAQGYKGANVKVAVLDTGIHAAHPDLNVAGGASFVPSEPNATQDFQSHGTHVAGTIAALDNTIGVLGVAPSASLYAVKVLDRNGDGQYSWIISGIEWAVANNMDVINMSLGGPDGSTALKNAVDTANKRGVVVVAAAGNSGSTGSTSTVGYPAKYDSTIAVANVNSSNVRNSSSSAGPELDVSAPGTSILSTVPSSGYTSYTGTSMASPHVAGAAALILSKNPNLSNSQVRQRLETTATPLGNSFYYGKGLINAEAASN

SEQ ID NO: 16 - protein, 275 aa, Artificial Sequence
  Mutante 15
AQTVPYGITQIKAPAVHAQGYKGANVKVAVLDTGIHAAHPDLNVAGGASFVPSEPNATQDFQSHGTHVAGTIAALDNTIGVLGVAPSASLYAVKVLDRNGDGQYSWIISGIEWAVANNMDVINMSLGGPDGSTALKNAVDTANKRGVVVVAAAGNSGSTGSTSTVGYPAKYDSTIAVANVNSSNVRNSSSSAGPELDVSAPGTSILSTVPSSGYTSYTGTSMASPHVAGAAALILSKNPNLSNSQVRQRLETTATPLGNSFYYGKGLINAEAASN

SEQ ID NO: 17 - protein, 275 aa, Artificial Sequence
  Mutante 16
AQTVPYGITQIKAPAVHAQGYKGANVKVAVLDTGIHAAHPDLNVAGGASFVPSEPNATQDFQSHGTHVAGTIAALDNTIGVLGVAPSASLYAVKVLDRNGDGQYSWIISGIEWAVANNMDVINMSLGGPDGSTALKNAVDTANKRGVVVVAAAGNGGSTGSTSTVGYPAKYDSTIAVANVNSSNVRNSSSSAGPELDVSAPGTSILSTVPSSGYTSYTGTSMASPHVAGAAALILSKNPNLSNSQVRQRLETTATPLGNSFYYGKGLINAEAASN

SEQ ID NO: 18 - protein, 275 aa, Artificial Sequence
  Mutante 17
AQTVPYGITQIKAPAVHAQGYKGANVKVAVLDTGIHAAHPDLNVAGGASFVPSEPNATQDFQSHGTHVAGTIAALDNTIGVLGVAPSASLYAVKVLDRNGDGQYSWIISGIEWAVANNMDVINMSLGGPDGSTALKNAVDTANKRGVVVVAAAGNYGSTGSTSTVGYPAKYDSTIAVANVNSSNVRNSSSSAGPELDVSAPGTSILSTVPSSGYTSYTGTSMASPHVAGAAALILSKNPNLSNSQVRQRLETTATPLGNSFYYGKGLINAEAASN

SEQ ID NO: 19 - protein, 275 aa, Artificial Sequence
  Mutante 18
AQTVPYGITQIKAPAVHAQGYKGANVKVAVLDTGIHAAHPDLNVAGGASFVPSEPNATQDFQSHGTHVAGTIAALDNTIGVLGVAPSASLYAVKVLDRNGDGQYSWIISGIEWAVANNMDVINMSLGGPDGSTALKNAVDTANKRGVVVVAAAGNSGSTGSTSTVGYPAKYDSTIAVANVNSSNVRNSSSSAGPELDVSAPGTSILSTVPSSGYTSMTGTSMASPHVAGAAALILSKNPNLSNSQVRQRLETTATPLGNSFYYGKGLINAEAASN

SEQ ID NO: 20 - protein, 275 aa, Artificial Sequence
  Mutante 19
AQTVPYGITQIKAPAVHAQGYKGANVKVAVLDTGIHAAHPDLNVAGGASFVPSEPNATQDFQSHGTHVAGTIAALDNTIGVLGVAPSASLYAVKVLDRNGDGQYSWIISGIEWAVANNMDVINMSLGGPDGSTALKKAVDTANKRGVVVVAAAGNSGSTGSTSTVGYPAKYDSTIAVANVNSSNVRNSSSSAGPELDVSAPGTSILSTVPSSGYTSYTGTSMASPHVAGAAALILSKNPNLSNSQVRQRLETTATPLGNSFYYGKGLINAEAASN

SEQ ID NO: 21 - protein, 275 aa, Artificial Sequence
  Mutante 20
AQTVPYGIPQIKAPAVHAQGYKGANVKVAVLDTGIHAAHPDLNVAGGASFVPSEPNATQDYQSHGTHVAGTIAALDNTIGVLGVAPSASLYSVKVLDRNGDGQYSWIISGIEWAVANNMDVINMSLGGPDGSTALKNAVDTANKRGVVVVAAAGNSGSTGSTSTVGYPAKYDSTIAVANVNSSNVRNSSSSAGPELDVSAPGTSILSTVPSSGYTSYTGTSMASPHVAGAAALILSKNPNLSNSQVRQRLETTATPLGNSFYYGKGLINAEAASN

SEQ ID NO: 22 - protein, 275 aa, Artificial Sequence
  Mutante 21^
AQTVPYGIPQIKAPAVHAQGYKGANVKVAVLDTGIHAAHPDLNVAGGASFVPSEPNATQDFQSHGTHVAGTIAALDNTIGVLGVAPSASLYAVKVLDRNGDGQYSWIISGIEWAVANNMDVINMSLGGPDGSTALKNAVDTANKRGVVVVAAAGNSGSTGSSSTVGYPAKYDSTIAVANVNSSNVRNSSSSAGPELDVSAPGTSILSTVPSSGYTSYTGTSMASPHVAGAAALILSKNPNLSNSQVRQRLETTATPLGNSFYYGKGLINAEAASN

SEQ ID NO: 23 - protein, 275 aa, Artificial Sequence
  Mutante 22
AQTVPYGIPQIKAPAVHAQGYKGANVKVAVLDTGIHAAHPDLNVAGGASFVPSEPNATQDFQSHGTHVAGTIAALDNTIGVLGVAPSASLYAVKVLDRNGDGQYSWIISGIEWAVANNMDVINMSLGGPDGSTALKNAVDTANKRGVVVVAAAGNSGSTGSTSTVGYPAKYDSTIAVANVNSSNVRNSSSSVGPELDVSAPGTSILSTVPSSGYTSYTGTSMASPHVAGAAALILSKNPNLSNSQVRQRLETTATPLGNSFYYGKGLINAEAASN

SEQ ID NO: 24 - protein, 275 aa, Artificial Sequence
  Mutante 23
AQTVPYGIHQIKAPAVHDQGYKGANVKVAVLDTGIHAAHPDLNVAGGASFVPSEPNATQDFQSHGTHVAGTIAALDNTIGVLGVAPSASLYAVKVLDRNGDGQYSWIISGIEWAVANNMDVINMSLGGPDGSTALKNAVDTANKRGVVVVAAAGNSGSIGSTSTVGYPAKYDSTIAVANVNSSNVRNSSSSAGPELDVSAPGTSILSTVPSSGYTSYTGTSMASPHVAGAAALILSKNPNLSNSQVRQRLETTATPLGNSFYYGKGLINAEAASN

SEQ ID NO: 25 - protein, 275 aa, Artificial Sequence
  Mutante 24
AQTVPYGITQIKAPAVHAQGYKGANVKVAVLDTGIHAAHPDLNVAGGASFVPSEPNATQDFQSHGTHVAGTIAALDNTIGVLGVAPSASLYAVKVLDRNGDGQYSWIISGIEWAVANNMDVINMSLGGPNGSTALKNAVDTANNRGVVVVAAAGNSGSTGSTSTVGYPAKYGSTIAVANVNSSNVRNSSSSAGPELDVSAPGTSILSTVPSSGYTSYTGTSMASPHVAGAAALILSKNPNLSNSQVRQRLENTATPLGNSFYYGKGLINAEAASN